European Patent Application EP 4 327 659 A2, published February 28, 2024. Title: MICROBIAL INOCULANTS AND METHODS. Applicant: CERAGEN INC. The sequence listing filed with the application follows.

SEQUENCE LISTING (5 sequences)

SEQ ID NO: 1 - DNA, 1504 bp, Rhodococcus erythropolis
  source 1..1504: mol_type = genomic DNA
tttgatcctggctcaggacgaacgctggcggcgtgcttaacacatgcaagtcgagcggtaaggcctttcggggtacacgagcggcgaacgggtgagtaacacgtgggtgatctgccctgcacttcgggataagcctgggaaactgggtctaataccggatatgacctcctatcgcatggtgggtggtggaaagatttatcggtgcaggatgggcccgcggcctatcagcttgttggtggggtaatggcctaccaaggcgacgacgggtagccgacctgagagggtgaccggccacactgggactgagacacggcccagactcctacgggaggcagcagtggggaatattgcacaatgggcgaaagcctgatgcagcgacgccgcgtgagggatgacggccttcgggttgtaaacctctttcagcagggacgaagcgcaagtgacggtacctgcagaagaagcaccggctaactacgtgccagcagccgcggtaatacgtagggtgcaagcgttgtccggaattactgggcgtaaagagttcgtaggcggtttgtcgcgtcgtttgtgaaaaccagcagctcaactgctggcttgcaggcgatacgggcagacttgagtactgcaggggagactggaattcctggtgtagcggtgaaatgcgcagatatcaggaggaacaccggtggcgaaggcgggtctctgggcagtaactgacgctgaggaacgaaagcgtgggtagcgaacaggattagataccctggtagtccacgccgtaaacggtgggcgctaggtgtgggttccttccacggaatccgtgccgtagctaacgcattaagcgccccgcctggggagtacggccgcaaggctaaaactcaaaggaattgacgggggcccgcacaagcggcggagcatgtggattaattcgatgcaacgcgaagaaccttacctgggtttgacatataccggaaagctgcagagatgtggccccccttgtggtcggtatacaggtggtgcatggctgtcgtcagctcgtgtcgtgagatgttgggttaagtcccgcaacgagcgcaacccctatcttatgttgccagcacgttatggtggggactcgtaagagactgccggggtcaactcggaggaaggtggggacgacgtcaagtcatcatgccccttatgtccagggcttcacacatgctacaatggccagtacagagggctgcgagaccgtgaggtggagcgaatcccttaaagctggtctcagttcggatcggggtctgcaactcgaccccgtgaagtcggagtcgctagtaatcgcagatcagcaacgctgcggtgaatacgttcccgggccttgtacacaccgcccgtcacgtcatgaaagtcggtaacacccgaagccggtggcttaaccccttgtgggagggagccgtcgaaggtgggatcggcgattgggacgaagtcgtaacaaggtagccgtaccggaaggtgcggctggatcacctcc

SEQ ID NO: 2 - DNA, 1538 bp, Serratia grimesii
  source 1..1538: mol_type = genomic DNA
ttgaagagtttgatcatggctcagattgaacgctggcggcaggcctaacacatgcaagtcgagcggtagcacaagagagcttgctctctgggtgacgagcggcggacgggtgagtaatgtctgggaaactgcctgatggagggggataactactggaaacggtagctaataccgcataacgtcttcggaccaaagtgggggaccttcgggcctcacgccatcagatgtgcccagatgggattagctagtaggtggggtaatggctcacctaggcgacgatccctagctggtctgagaggatgaccagccacactggaactgagacacggtccagactcctacgggaggcagcagtggggaatattgcacaatgggcgcaagcctgatgcagccatgccgcgtgtgtgaagaaggccttcgggttgtaaagcactttcagcgaggaggaagggtagtgtgttaatagcacattgcattgacgttactcgcagaagaagcaccggctaactccgtgccagcagccgcggtaatacggagggtgcaagcgttaatcggaattactgggcgtaaagcgcacgcaggcggtttgttaagtcagatgtgaaatccccgcgcttaacgtgggaactgcatttgaaactggcaagctagagtcttgtagaggggggtagaattccaggtgtagcggtgaaatgcgtagagatctggaggaataccggtggcgaaggcggccccctggacaaagactgacgctcaggtgcgaaagcgtggggagcaaacaggattagataccctggtagtccacgctgtaaacgatgtcgacttggaggttgtgcccttgaggcgtggcttccggagctaacgcgttaagtcgaccgcctggggagtacggccgcaaggttaaaactcaaatgaattgacgggggcccgcacaagcggtggagcatgtggtttaattcgatgcaacgcgaagaaccttacctactcttgacatccagagaattcgctagagatagcttagtgccttcgggaactctgagacaggtgctgcatggctgtcgtcagctcgtgttgtgaaatgttgggttaagtcccgcaacgagcgcaacccttatcctttgttgccagcacgtaatggtgggaactcaaaggagactgccggtgataaaccggaggaaggtggggatgacgtcaagtcatcatggcccttacgagtagggctacacacgtgctacaatggcgtatacaaagagaagcgaactcgcgagagcaagcggacctcataaagtacgtcgtagtccggatcggagtctgcaactcgactccgtgaagtcggaatcgctagtaatcgtagatcagaatgctacggtgaatacgttcccgggccttgtacacaccgcccgtcacaccatgggagtgggttgcaaaagaagtaggtagcttaaccttcgggagggcgcttaccactttgtgattcatgactggggtgaagtcgtaacaaggtaaccgtaggggaacctgcggttggatcacctcct

SEQ ID NO: 3 - DNA, 1540 bp, Stenotrophomonas maltophilia
  source 1..1540: mol_type = genomic DNA
tgaagagtttgatcctggctcagagtgaacgctggcggtaggcctaacacatgcaagtcgaacggcagcacagaggagcttgctccttgggtggcgagtggcggacgggtgaggaatacatcggaatctactttttcgtgggggataacgtagggaaacttacgctaataccgcatacgacctacgggtgaaagcaggggatcttcggaccttgcgcgattgaatgagccgatgtcggattagctagttggcggggtaaaggcccaccaaggcgacgatccgtagctggtctgagaggatgatcagccacactggaactgagacacggtccagactcctacgggaggcagcagtggggaatattggacaatgggcgcaagcctgatccagccataccgcgtgggtgaagaaggccttcgggttgtaaagcccttttgttgggaaagaaatccagccggctaatacctggttgggatgacggtacccaaagaataagcaccggctaacttcgtgccagcagccgcggtaatacgaagggtgcaagcgttactcggaattactgggcgtaaagcgtgcgtaggtggttatttaagtccgttgtgaaagccctgggctcaacctgggaactgcagtggatactggatgactagaatgtggtagagggtagcggaattcctggtgtagcagtgaaatgcgtagagatcaggaggaacatccatggcgaaggcagctacctggaccaacattgacactgaggcacgaaagcgtggggagcaaacaggattagataccctggtagtccacgccctaaacgatgcgaactggatgttgggtgcaatttggcacgcagtatcgaagctaacgcgttaagttcgccgcctggggagtacggtcgcaagactgaaactcaaaggaattgacgggggcccgcacaagcggtggagtatgtggtttaattcgatgcaacgcgaagaaccttacctggccttgacatgtcgagaactttccagagatggatgggtgccttcgggaactcgaacacaggtgctgcatggctgtcgtcagctcgtgtcgtgagatgttgggttaagtcccgcaacgagcgcaacccttgtccttagttgccagcacgtaatggtgggaactctaaggagaccgccggtgacaaaccggaggaaggtggggatgacgtcaagtcatcatggcccttacggccagggctacacacgtactacaatggtagggacagagggctgcaagccggcgacggtaagccaatcccagaaaccctatctcagtccggattggagtctgcaactcgactccatgaagtcggaatcgctagtaatcgcagatcagcattgctgcggtgaatacgttcccgggccttgtacacaccgcccgtcacaccatgggagtttgttgcaccagaagcaggtagcttaaccttcgggagggcgcttgccacggtgtggccgatgactggggtgaagtcgtaacaaggtagccgtatcggaaggtgcggctggatcacctcctt

SEQ ID NO: 4 - DNA, 1531 bp, Pseudomonas toyotomiensis
  source 1..1531: mol_type = genomic DNA
tgaagagtttgatcatggctcagattgaacgctggcggcaggcctaacacatgcaagtcgagcggatgaggggagcttgctccctgatttagcggcggacgggtgagtaatgcctaggaatctgcctagtggtgggggataacgttccgaaaggaacgctaataccgcatacgtcctacgggagaaagcgggggatcttcggacctcgcgccattagatgagcctaggtcggattagctagttggtgaggtaaaggctcaccaaggcgacgatccgtaactggtctgagaggatgatcagtcacactggaactgagacacggtccagactcctacgggaggcagcagtggggaatattggacaatgggcgaaagcctgatccagccatgccgcgtgtgtgaagaaggtcttcggattgtaaagcactttaagttgggaggaagggtattcacctaatacgtgagtattttgacgttaccgacagaataagcaccggctaacttcgtgccagcagccgcggtaatacgaagggtgcaagcgttaatcggaattactgggcgtaaagcgcgcgtaggtggttcgttaagttggatgtgaaagccccgggctcaacctgggaactgcatccaaaactggcgagctagagtacggtagagggtggtggaatttcctgtgtagcggtgaaatgcgtagatataggaaggaacaccagtggcgaaggcgaccacctggactgatactgacactgaggtgcgaaagcgtggggagcaaacaggattagataccctggtagtccacgccgtaaacgatgtcaactagccgttggaatccttgagattttagtggcgcagctaacgcattaagttgaccgcctggggagtacggccgcaaggttaaaactcaaatgaattgacgggggcccgcacaagcggtggagcatgtggtttaattcgaagcaacgcgaagaaccttacctggccttgacatgctgagaactttccagagatggattggtgccttcgggaactcagacacaggtgctgcatggctgtcgtcagctcgtgtcgtgagatgttgggttaagtcccgtaacgagcgcaacccttgtccttagttaccagcacgttatggtgggcactctaaggagactgccggtgacaaaccggaggaaggtggggatgacgtcaagtcatcatggcccttacggccagggctacacacgtgctacaatggtcggtacaaagggttgccaagccgcgaggtggagctaatcccataaaaccgatcgtagtccggatcgcagtctgcaactcgactgcgtgaagtcggaatcgctagtaatcgtgaatcagaatgtcacggtgaatacgttcccgggccttgtacacaccgcccgtcacaccatgggagtgggttgctccagaagtagctagtctaaccttcggggggacggttaccacggagtgattcatgactggggtgaagtcgtaacaaggtagccgtaggggaacctgcggctggatcacctcct

SEQ ID NO: 5 - DNA, 1471 bp, Shinella zoogloeoides
  source 1..1471: mol_type = genomic DNA
tttgatcctggctcagaacgaacgctggcggcaggcttaacacatgcaagtcgaacgccccgcaaggggagtggcagacgggtgagtaacgcgtgggaatctacccatctctacggaataactcagggaaacttgtgctaataccgtatacgcccttcgggggaaagatttatcggagatggatgagcccgcgttggattagctagttggtggggtaaaggcctaccaaggcgacgatccatagctggtctgagaggatgatcagccacattgggactgagacacggcccaaactcctacgggaggcagcagtggggaatattggacaatgggcgcaagcctgatccagccatgccgcgtgagtgatgaaggccctagggttgtaaagctctttcaccggtgaagataatgacggtaaccggagaagaagccccggctaacttcgtgccagcagccgcggtaatacgaagggggctagcgttgttcggaattactgggcgtaaagcgcacgtaggcgggtatttaagtcaggggtgaaatcccagagctcaactctggaactgcctttgatactgggtacctagagtatggaagaggtaagtggaattccgagtgtagaggtgaaattcgtagatattcggaggaacaccagtggcgaaggcggcttactggtccattactgacgctgaggtgcgaaagcgtggggagcaaacaggattagataccctggtagtccacgccgtaaacgatgaatgttagccgtcggcatgcatgcatgtcggtggcgcagctaacgcattaaacattccgcctggggagtacggtcgcaagattaaaactcaaaggaattgacgggggcccgcacaagcggtggagcatgtggtttaattcgaagcaacgcgcagaaccttaccagcccttgacatgtcggtcgcggattacagagatgttttccttcagttaggctggaccgaacacaggtgctgcatggctgtcgtcagctcgtgtcgtgagatgttgggttaagtcccgcaacgagcgcaaccctcgcccttagttgccagcattcagttgggcactctaaggggactgccggtgataagccgagaggaaggtggggatgacgtcaagtcctcatggcccttacgggctgggctacacacgtgctacaatggtggtgacagtgggcagcgagacagcgatgtcgagctaatctccaaaagccatctcagttcggattgcactctgcaactcgagtgcatgaagttggaatcgctagtaatcgcggatcagcatgccgcggtgaatacgttcccgggccttgtacacaccgcccgtcacaccatgggagttggttttacccgaaggcactgcgctaaccgcaagggggcaggtgaccacggtagggtcagcgactggggtgaagtcgtaacaaggtagccgtaggggaacctgcggctggatcacctcc